European Patent Specification EP 3 634 981 B1, published December 27, 2023. Title: LIPIDATED STREPTOCOCCUS PNEUMONIAE ANTIGEN COMPOSITIONS, METHODS OF PREPARATION AND USE. Applicant: National Research Council Of Canada National Health Research Institutes. Application 15/619,075. The sequence listing filed with the application follows.

SEQUENCE LISTING (9 sequences)

SEQ ID NO: 1 - protein, 309 aa, Streptococcus pneumoniae
MKKLGTLLVLFLSAIILVACASGKKDTTSGQKLKVVATNSIIADITKNIAGDKIDLHSIVPIGQDPHEYEPLPEDVKKTSEADLIFYNGINLETGGNAWFTKLVENAKKTENKDYFAVSDGVDVIYLEGQNEKGKEDPHAWLNLENGIIFAKNIAKQLSAKDPNNKEFYEKNLKEYTDKLDKLDKESKDKFNKIPAEKKLIVTSEGAFKYFSKAYGVPSAYIWEINTEEEGTPEQIKTLVEKLRQTKVPSLFVESSVDDRPMKTVSQDTNIPIYAQIFTDSIAEQGKEGDSYYSMMKYNLDKIAEGLAK

SEQ ID NO: 2 - protein, 290 aa, Streptococcus pneumoniae
MASGKKDTTSGQKLKVVATNSIIADITKNIAGDKIDLHSIVPIGQDPHEYEPLPEDVKKTSEADLIFYNGINLETGGNAWFTKLVENAKKTENKDYFAVSDGVDVIYLEGQNEKGKEDPHAWLNLENGIIFAKNIAKQLSAKDPNNKEFYEKNLKEYTDKLDKLDKESKDKFNKIPAEKKLIVTSEGAFKYFSKAYGVPSAYIWEINTEEEGTPEQIKTLVEKLRQTKVPSLFVESSVDDRPMKTVSQDTNIPIYAQIFTDSIAEQGKEGDSYYSMMKYNLDKIAEGLAK

SEQ ID NO: 3 - protein, 379 aa, Streptococcus pneumoniae
MEESPVASQSKAEKDYDAAKKDAKNAKKAVEDAQKALDDAKAAQKKYDEDQKKTEEKAALEKAASEEMDKAVAAVQQAYLAYQQATDKAAKDAADKMIDEAKKREEEAKTKFNTVRAMVVPEPEQLAETKKKSEEAKQKAPELTKKLEEAKAKLEEAEKKATEAKQKVDAEEVAPQAKIAELENQVHRLEQELKEIDESESEDYAKEGFRAPLQSKLDAKKAKLSKLEELSDKIDELDAEIAKLEDQLKAAEENNNVEDYFKEGLEKTIAAKKAELEKTEADLKKAVNEPEKPAPAPETPAPEAPAEQPKPAPAPQPAPAPKPEKPAEQPKPEKTDDQQAEEDYARRSEEEYNRLTQQQPPKAEKPAPAPKLEHHHHHH

SEQ ID NO: 4 - protein, 490 aa, Streptococcus pneumoniae
MFASKSERKVHYSIRKFSIGVASVAVASLVMGSVVHATENEGSTQAATSSNMAKTEHRKAAKQVVDEYIEKMLREIQLDRRKHTQNVALNIKLSAIKTKYLRELNVLEEKSKDELPSEIKAKLDAAFEKFKKDTLKPGEKVAEAKKKVEEAKKKAEDQKEEDRRNYPTNTYKTLELEIAEFDVKVKEAELELVKEEAKESRNEGTIKQAKEKVESKKAEATRLENIKTDRKKAEEEAKRKADAKLKEANVATSDQGKPKGRAKRGVPGELATPDKKENDAKSSDSSVGEETLPSSSLKSGKKVAEAEKKVEEAEKKAKDQKEEDRRNYPTNTYKTLDLEIAESDVKVKEAELELVKEEAKEPRDEEKIKQAKAKVESKKAEATRLENIKTDRKKAEEEAKRKAAEEDKVKEKPAEQPQPAPATQPEKPAPKPEKPAEQPKAEKTDDQQAEEDYARRSEEEYNRLTQQQPPKTEKPAQPSTPKLEHHHHHH

SEQ ID NO: 5 - protein, 20 aa, Streptococcus pneumoniae
MKKLGTLLVLFLSAIILVAC

SEQ ID NO: 6 - DNA, 954 bp, Streptococcus pneumoniae
atgaaaaaactgggcaccctgctggtgctgtttctgagcgcgattattctggtggcgtgcgcgagcggcaaaaaagataccaccagcggccagaaactgaaagtggtggcgaccaacagcattattgcggatattaccaaaaacattgcgggcgataaaattgatctgcatagcattgtgccgattggccaggatccgcatgaatatgaaccgctgccggaagatgtgaaaaaaaccagcgaagcggatctgattttttataacggcattaacctggaaaccggcggcaacgcgtggtttaccaaactggtggaaaacgcgaaaaaaaccgaaaacaaagattattttgcggtgagcgatggcgtggatgtgatttatctggaaggccagaacgaaaaaggcaaagaagatccgcatgcgtggctgaacctggaaaacggcattatttttgcgaaaaacattgcgaaacagctgagcgcgaaagatccgaacaacaaagaattttatgaaaaaaacctgaaagaatataccgataaactggataaactggataaagaaagcaaagataaatttaacaaaattccggcggaaaaaaaactgattgtgaccagcgaaggcgcgtttaaatattttagcaaagcgtatggcgtgccgagcgcgtatatttgggaaattaacaccgaagaagaaggcaccccggaacagattaaaaccctggtggaaaaactgcgtcagaccaaagtgccgagcctgtttgtggaaagcagcgtggatgatcgtccgatgaaaaccgtgagccaggataccaacattccgatttatgcgcagatttttaccgatagcattgcggaacagggcaaagaaggcgatagctattatagcatgatgaaatataacctggataaaattgcggaaggcctggcgaaactcgagcaccaccaccaccaccactga

SEQ ID NO: 7 - protein, 315 aa, Streptococcus pneumoniae
MKKLGTLLVLFLSAIILVACASGKKDTTSGQKLKVVATNSIIADITKNIAGDKIDLHSIVPIGQDPHEYEPLPEDVKKTSEADLIFYNGINLETGGNAWFTKLVENAKKTENKDYFAVSDGVDVIYLEGQNEKGKEDPHAWLNLENGIIFAKNIAKQLSAKDPNNKEFYEKNLKEYTDKLDKLDKESKDKFNKIPAEKKLIVTSEGAFKYFSKAYGVPSAYIWEINTEEEGTPEQIKTLVEKLRQTKVPSLFVESSVDDRPMKTVSQDTNIPIYAQIFTDSIAEQGKEGDSYYSMMKYNLDKIAEGLAKHHHHHH

SEQ ID NO: 8 - protein, 296 aa, Streptococcus pneumoniae
MASGKKDTTSGQKLKVVATNSIIADITKNIAGDKIDLHSIVPIGQDPHEYEPLPEDVKKTSEADLIFYNGINLETGGNAWFTKLVENAKKTENKDYFAVSDGVDVIYLEGQNEKGKEDPHAWLNLENGIIFAKNIAKQLSAKDPNNKEFYEKNLKEYTDKLDKLDKESKDKFNKIPAEKKLIVTSEGAFKYFSKAYGVPSAYIWEINTEEEGTPEQIKTLVEKLRQTKVPSLFVESSVDDRPMKTVSQDTNIPIYAQIFTDSIAEQGKEGDSYYSMMKYNLDKIAEGLAKHHHHHH

SEQ ID NO: 9 - protein, 290 aa, Streptococcus pneumoniae
CASGKKDTTSGQKLKVVATNSIIADITKNIAGDKIDLHSIVPIGQDPHEYEPLPEDVKKTSEADLIFYNGINLETGGNAWFTKLVENAKKTENKDYFAVSDGVDVIYLEGQNEKGKEDPHAWLNLENGIIFAKNIAKQLSAKDPNNKEFYEKNLKEYTDKLDKLDKESKDKFNKIPAEKKLIVTSEGAFKYFSKAYGVPSAYIWEINTEEEGTPEQIKTLVEKLRQTKVPSLFVESSVDDRPMKTVSQDTNIPIYAQIFTDSIAEQGKEGDSYYSMMKYNLDKIAEGLAK